European Patent Application EP 4 512 893 A1, published February 26, 2025. Title: Fructanase variant. Applicant: AB Enzymes Oy. The sequence listing filed with the application follows.

SEQUENCE LISTING (13 sequences)

SEQ ID NO: 1 - protein, 1279 aa, Lactobacillus crispatus
DTQSPVNIEQKNKSAELIKQNSDISTSAQQHNKNANGKTEDTSTQSTSTDLQNTNGKTEDTSTQSTSTDLQNTNTQKSFKNQSQEPESSTKAGEVKTLKDFTFSQNGKWSEQKDGIHSDARGQGDSFAYTKVKGDNFMYSADVVFQTNQGAAAITFRDNNDPDNKDGYAVNVDASSHKAKFWRWHDNKDYQLIDERDVKQTADNTYNLKVVANGHWLEYFVNDVLVASNGDYTLQKGDKGQPSVTNNGYFGLLNWNSNVIFKNVKYTKLDQSFTPLVSDITVTSDKGKVEEKGQFSPEQPIYIQYVDNDASTVNLKVKTDSPKAKVVAYDLNNNAYTDLKNIPVQVGANYLTVVSEVTASDGTKVESVYRINVHRLHPNENYYNELYRDQYHFSVKEGWSNDPNGLVYFNGKYHMFYQFYDDTIWGPMHWAHATSKDLIHWKNEPIALYPDANGAMFSGSIVVDKGNTSGLFDNDKGGLVALVTTDGNGQRIELAYSRDEGKTWDKLPNLVADWQKDPLQVQDFRDPKVFRWNDKWFMVLAGGPLRIYSSTNLQNWQVESEYSNINTECPDLYPIRANDGQLKWVLSRGGRFYKIGDFKEVNGKWSFIPDEAYKDQDGIMNFGKDSYAAMTYYQHSFGTEKDPTLPDIIEENWMNNWDYCNLVGNTVGQSFNGTYNLNLKVGLVKDGDKYLLTQTPIKAYEALRDNAHKVEYKDVTVTPNNDLFKNFKGDSYEIVSTFRPSKSTTKVGFNVRVGKGQATKVIYDLTTNKIYIDRSKSGVQINNKFSELNEQPVTRNADGSISLHLYVDRASVEAFTKGDTVLGANQIFPAPQSLGLQVVSEGGDSKADITLYPIKSVWTDKQKVNKPLEIVQVSPKEVRLNVGDSTTLTAYVMPGNVSQALDWSINDESLASITKDPESNSLKIVAKKAGTLTVTVKSHEDPSLSKTYKITILKNNFKTNIKDLKPLSGNWYVDDQDLHDENVSSNDYIMSPTKVSSSEYDMNLDVKYQKGLVNIFFASANEDPNGAYSLQLGGDKTLRLFRFYGDTITTTDLPAALNDGKLHHVAIHKTQNAVKVTIDGKEAMDYTFDKVDPGFNSAYVGLGLWDGAADFQNLYVKAATENDDNSSSSIDFNDQEIPNVSTDDNNSIIEKPSETVKTVVFTAKSLMHNAFVYDNQGKRIEKIVLKAGSVLKVGHIKLINHKRYYQLDNGKYIKAGNIDAYVRKLRRNAFVYNRAGKHIKKSLIRKGKKVKTYGSPVVIKGIKYYIVGNNRYIKAVNFM

SEQ ID NO: 2 - protein, 1279 aa, synthetic construct
DTQSPVNIEQKNKSAELIKQNSDISTSAQQHNKNANGKTEDTSTQSTSTDLQNTNGKTEDTSTQSTSTDLQNTNTQKSFKNQSQEPESSTKAGEVKTLKDFTFSQNGKWSEQKDGIHSDARGQGDSFAYTKVKGDNFMYSADVVFQTNQGAAAITFRDNNDPDNKDGYAVNVDASSHKAKFWRWHDNKDYQLIDERDVKQTADNTYNLKVVANGHWLEYFVNDVLVASNGDYTLQKGDKGQPSVTNNGYFGLLNWNSNVIFKNVKYTKLDQSFTPLVSDITVTSDKGKVEEKGQFSPEQPIYIQYVDNDASTVNLKVKTDSPKAKVVAYDLNNNAYTDLKNIPVQVGANYLTVVSEVTASDGTKVESVYRINVHRLHPNENYYNELYRDQYHFSVKEGWSNDPNGLVYFNGKYHMFYQFYDDTIWGPMHWAHATSKDLIHWKNEPIALYPDANGAMFSGSIVVDKGNTSGLFDNDKGGLVALVTTDGNGQRIELAYSRDEGKTWDKLPNLVADWQKDPLQVQDFRDPKVFRWNDKWFMVLAGGPLRIYSSTNLQNWQVESEYSNINTECPDLYPIRANDGQLKWVLSRGGRFYKIGDFKEVNGKWSFIPDEAYKDQDGIMNFGKDSYAAMTYYQHSFGTEKDPTLPDIIEENWMNNWDYCNLVGNTVGQSFNGAYNLNLKVGLVKDGDKYLLTQTPIKAYEALRDNAHKVEYKDVTVTPNNDLFKNFKGDSYEIVSTFRPSKSTTKVGFNVRVGKGQATKVIYDLTTNKIYIDRSKSGVQINNKFSELNEQPVTRNADGSISLHLYVDRASVEAFTKGDTVLGANQIFPAPQSLGLQVVSEGGDSKADITLYPIKSVWTDKQKVNKPLEIVQVSPKEVRLNVGDSTTLTAYVMPGNVSQALDWSINDESLASITKDPESNSLKIVAKKAGTLTVTVKSHEDPSLSKTYKITILKNNFKTNIKDLKPLSGNWYVDDQDLHDENVSSNDYIMSPTKVSSSEYDMNLDVKYQKGLVNIFFASANEDPNGAYSLQLGGDKTLRLFRFYGDTITTTDLPAALNDGKLHHVAIHKTQNAVKVTIDGKEAMDYTFDKVDPGFNSAYVGLGLWDGAADFQNLYVKAATENDDNSSSSIDFNDQEIPNVSTDDNNSIIEKPSETVKTVVFTAKSLMHNAFVYDNQGKRIEKIVLKAGSVLKVGHIKLINHKRYYQLDNGKYIKAGNIDAYVRKLRRNAFVYNRAGKHIKKSLIRKGKKVKTYGSPVVIKGIKYYIVGNNRYIKAVNFM

SEQ ID NO: 3 - protein, 1165 aa, synthetic construct
DTQSPVNIEQKNKSAELIKQNSDISTSAQQHNKNANGKTEDTSTQSTSTDLQNTNGKTEDTSTQSTSTDLQNTNTQKSFKNQSQEPESSTKAGEVKTLKDFTFSQNGKWSEQKDGIHSDARGQGDSFAYTKVKGDNFMYSADVVFQTNQGAAAITFRDNNDPDNKDGYAVNVDASSHKAKFWRWHDNKDYQLIDERDVKQTADNTYNLKVVANGHWLEYFVNDVLVASNGDYTLQKGDKGQPSVTNNGYFGLLNWNSNVIFKNVKYTKLDQSFTPLVSDITVTSDKGKVEEKGQFSPEQPIYIQYVDNDASTVNLKVKTDSPKAKVVAYDLNNNAYTDLKNIPVQVGANYLTVVSEVTASDGTKVESVYRINVHRLHPNENYYNELYRDQYHFSVKEGWSNDPNGLVYFNGKYHMFYQFYDDTIWGPMHWAHATSKDLIHWKNEPIALYPDANGAMFSGSIVVDKGNTSGLFDNDKGGLVALVTTDGNGQRIELAYSRDEGKTWDKLPNLVADWQKDPLQVQDFRDPKVFRWNDKWFMVLAGGPLRIYSSTNLQNWQVESEYSNINTECPDLYPIRANDGQLKWVLSRGGRFYKIGDFKEVNGKWSFIPDEAYKDQDGIMNFGKDSYAAMTYYQHSFGTEKDPTLPDIIEENWMNNWDYCNLVGNTVGQSFNGTYNLNLKVGLVKDGDKYLLTQTPIKAYEALRDNAHKVEYKDVTVTPNNDLFKNFKGDSYEIVSTFRPSKSTTKVGFNVRVGKGQATKVIYDLTTNKIYIDRSKSGVQINNKFSELNEQPVTRNADGSISLHLYVDRASVEAFTKGDTVLGANQIFPAPQSLGLQVVSEGGDSKADITLYPIKSVWTDKQKVNKPLEIVQVSPKEVRLNVGDSTTLTAYVMPGNVSQALDWSINDESLASITKDPESNSLKIVAKKAGTLTVTVKSHEDPSLSKTYKITILKNNFKTNIKDLKPLSGNWYVDDQDLHDENVSSNDYIMSPTKVSSSEYDMNLDVKYQKGLVNIFFASANEDPNGAYSLQLGGDKTLRLFRFYGDTITTTDLPAALNDGKLHHVAIHKTQNAVKVTIDGKEAMDYTFDKVDPGFNSAYVGLGLWDGAADFQNLYVKAATENDDNSSSSIDFNDQEIPNVSTDDNNSIIEKPSETVKTVVFTAKS

SEQ ID NO: 4 - protein, 1165 aa, synthetic construct
DTQSPVNIEQKNKSAELIKQNSDISTSAQQHNKNANGKTEDTSTQSTSTDLQNTNGKTEDTSTQSTSTDLQNTNTQKSFKNQSQEPESSTKAGEVKTLKDFTFSQNGKWSEQKDGIHSDARGQGDSFAYTKVKGDNFMYSADVVFQTNQGAAAITFRDNNDPDNKDGYAVNVDASSHKAKFWRWHDNKDYQLIDERDVKQTADNTYNLKVVANGHWLEYFVNDVLVASNGDYTLQKGDKGQPSVTNNGYFGLLNWNSNVIFKNVKYTKLDQSFTPLVSDITVTSDKGKVEEKGQFSPEQPIYIQYVDNDASTVNLKVKTDSPKAKVVAYDLNNNAYTDLKNIPVQVGANYLTVVSEVTASDGTKVESVYRINVHRLHPNENYYNELYRDQYHFSVKEGWSNDPNGLVYFNGKYHMFYQFYDDTIWGPMHWAHATSKDLIHWKNEPIALYPDANGAMFSGSIVVDKGNTSGLFDNDKGGLVALVTTDGNGQRIELAYSRDEGKTWDKLPNLVADWQKDPLQVQDFRDPKVFRWNDKWFMVLAGGPLRIYSSTNLQNWQVESEYSNINTECPDLYPIRANDGQLKWVLSRGGRFYKIGDFKEVNGKWSFIPDEAYKDQDGIMNFGKDSYAAMTYYQHSFGTEKDPTLPDIIEENWMNNWDYCNLVGNTVGQSFQGTYNLNLKVGLVKDGDKYLLTQTPIKAYEALRDNAHKVEYKDVTVTPNNDLFKNFKGDSYEIVSTFRPSKSTTKVGFNVRVGKGQATKVIYDLTTNKIYIDRSKSGVQINNKFSELNEQPVTRNADGSISLHLYVDRASVEAFTKGDTVLGANQIFPAPQSLGLQVVSEGGDSKADITLYPIKSVWTDKQKVNKPLEIVQVSPKEVRLNVGDSTTLTAYVMPGNVSQALDWSINDESLASITKDPESNSLKIVAKKAGTLTVTVKSHEDPSLSKTYKITILKNNFKTNIKDLKPLSGNWYVDDQDLHDENVSSNDYIMSPTKVSSSEYDMNLDVKYQKGLVNIFFASANEDPNGAYSLQLGGDKTLRLFRFYGDTITTTDLPAALNDGKLHHVAIHKTQNAVKVTIDGKEAMDYTFDKVDPGFNSAYVGLGLWDGAADFQNLYVKAATENDDNSSSSIDFNDQEIPNVSTDDNNSIIEKPSETVKTVVFTAKS

SEQ ID NO: 5 - protein, 1165 aa, synthetic construct
DTQSPVNIEQKNKSAELIKQNSDISTSAQQHNKNANGKTEDTSTQSTSTDLQNTNGKTEDTSTQSTSTDLQNTNTQKSFKNQSQEPESSTKAGEVKTLKDFTFSQNGKWSEQKDGIHSDARGQGDSFAYTKVKGDNFMYSADVVFQTNQGAAAITFRDNNDPDNKDGYAVNVDASSHKAKFWRWHDNKDYQLIDERDVKQTADNTYNLKVVANGHWLEYFVNDVLVASNGDYTLQKGDKGQPSVTNNGYFGLLNWNSNVIFKNVKYTKLDQSFTPLVSDITVTSDKGKVEEKGQFSPEQPIYIQYVDNDASTVNLKVKTDSPKAKVVAYDLNNNAYTDLKNIPVQVGANYLTVVSEVTASDGTKVESVYRINVHRLHPNENYYNELYRDQYHFSVKEGWSNDPNGLVYFNGKYHMFYQFYDDTIWGPMHWAHATSKDLIHWKNEPIALYPDANGAMFSGSIVVDKGNTSGLFDNDKGGLVALVTTDGNGQRIELAYSRDEGKTWDKLPNLVADWQKDPLQVQDFRDPKVFRWNDKWFMVLAGGPLRIYSSTNLQNWQVESEYSNINTECPDLYPIRANDGQLKWVLSRGGRFYKIGDFKEVNGKWSFIPDEAYKDQDGIMNFGKDSYAAMTYYQHSFGTEKDPTLPDIIEENWMNNWDYCNLVGNTVGQSFNGAYNLNLKVGLVKDGDKYLLTQTPIKAYEALRDNAHKVEYKDVTVTPNNDLFKNFKGDSYEIVSTFRPSKSTTKVGFNVRVGKGQATKVIYDLTTNKIYIDRSKSGVQINNKFSELNEQPVTRNADGSISLHLYVDRASVEAFTKGDTVLGANQIFPAPQSLGLQVVSEGGDSKADITLYPIKSVWTDKQKVNKPLEIVQVSPKEVRLNVGDSTTLTAYVMPGNVSQALDWSINDESLASITKDPESNSLKIVAKKAGTLTVTVKSHEDPSLSKTYKITILKNNFKTNIKDLKPLSGNWYVDDQDLHDENVSSNDYIMSPTKVSSSEYDMNLDVKYQKGLVNIFFASANEDPNGAYSLQLGGDKTLRLFRFYGDTITTTDLPAALNDGKLHHVAIHKTQNAVKVTIDGKEAMDYTFDKVDPGFNSAYVGLGLWDGAADFQNLYVKAATENDDNSSSSIDFNDQEIPNVSTDDNNSIIEKPSETVKTVVFTAKS

SEQ ID NO: 6 - protein, 1165 aa, synthetic construct
DTQSPVNIEQKNKSAELIKQNSDISTSAQQHNKNANGKTEDTSTQSTSTDLQNTNGKTEDTSTQSTSTDLQNTNTQKSFKNQSQEPESSTKAGEVKTLKDFTFSQNGKWSEQKDGIHSDARGQGDSFAYTKVKGDNFMYSADVVFQTNQGAAAITFRDNNDPDNKDGYAVNVDASSHKAKFWRWHDNKDYQLIDERDVKQTADNTYNLKVVANGHWLEYFVNDVLVASNGDYTLQKGDKGQPSVTNNGYFGLLNWNSNVIFKNVKYTKLDQSFTPLVSDITVTSDKGKVEEKGQFSPEQPIYIQYVDNDASTVNLKVKTDSPKAKVVAYDLNNNAYTDLKNIPVQVGANYLTVVSEVTASDGTKVESVYRINVHRLHPNENYYNELYRDQYHFSVKEGWSNDPNGLVYFNGKYHMFYQFYDDTIWGPMHWAHATSKDLIHWKNEPIALYPDANGAMFSGSIVVDKGNTSGLFDNDKGGLVALVTTDGNGQRIELAYSRDEGKTWDKLPNLVADWQKDPLQVQDFRDPKVFRWNDKWFMVLAGGPLRIYSSTNLQNWQVESEYSNINTECPDLYPIRANDGQLKWVLSRGGRFYKIGDFKEVNGKWSFIPDEAYKDQDGIMNFGKDSYAAMTYYQHSFGTEKDPTLPDIIEENWMNNWDYCNLVGNTVGQSFNGGYNLNLKVGLVKDGDKYLLTQTPIKAYEALRDNAHKVEYKDVTVTPNNDLFKNFKGDSYEIVSTFRPSKSTTKVGFNVRVGKGQATKVIYDLTTNKIYIDRSKSGVQINNKFSELNEQPVTRNADGSISLHLYVDRASVEAFTKGDTVLGANQIFPAPQSLGLQVVSEGGDSKADITLYPIKSVWTDKQKVNKPLEIVQVSPKEVRLNVGDSTTLTAYVMPGNVSQALDWSINDESLASITKDPESNSLKIVAKKAGTLTVTVKSHEDPSLSKTYKITILKNNFKTNIKDLKPLSGNWYVDDQDLHDENVSSNDYIMSPTKVSSSEYDMNLDVKYQKGLVNIFFASANEDPNGAYSLQLGGDKTLRLFRFYGDTITTTDLPAALNDGKLHHVAIHKTQNAVKVTIDGKEAMDYTFDKVDPGFNSAYVGLGLWDGAADFQNLYVKAATENDDNSSSSIDFNDQEIPNVSTDDNNSIIEKPSETVKTVVFTAKS

SEQ ID NO: 7 - protein, 1165 aa, synthetic construct
DTQSPVNIEQKNKSAELIKQNSDISTSAQQHNKNANGKTEDTSTQSTSTDLQNTNGKTEDTSTQSTSTDLQNTNTQKSFKNQSQEPESSTKAGEVKTLKDFTFSQNGKWSEQKDGIHSDARGQGDSFAYTKVKGDNFMYSADVVFQTNQGAAAITFRDNNDPDNKDGYAVNVDASSHKAKFWRWHDNKDYQLIDERDVKQTADNTYNLKVVANGHWLEYFVNDVLVASNGDYTLQKGDKGQPSVTNNGYFGLLNWNSNVIFKNVKYTKLDQSFTPLVSDITVTSDKGKVEEKGQFSPEQPIYIQYVDNDASTVNLKVKTDSPKAKVVAYDLNNNAYTDLKNIPVQVGANYLTVVSEVTASDGTKVESVYRINVHRLHPNENYYNELYRDQYHFSVKEGWSNDPNGLVYFNGKYHMFYQFYDDTIWGPMHWAHATSKDLIHWKNEPIALYPDANGAMFSGSIVVDKGNTSGLFDNDKGGLVALVTTDGNGQRIELAYSRDEGKTWDKLPNLVADWQKDPLQVQDFRDPKVFRWNDKWFMVLAGGPLRIYSSTNLQNWQVESEYSNINTECPDLYPIRANDGQLKWVLSRGGRFYKIGDFKEVNGKWSFIPDEAYKDQDGIMNFGKDSYAAMTYYQHSFGTEKDPTLPDIIEENWMNNWDYCNLVGNTVGQSFNGVYNLNLKVGLVKDGDKYLLTQTPIKAYEALRDNAHKVEYKDVTVTPNNDLFKNFKGDSYEIVSTFRPSKSTTKVGFNVRVGKGQATKVIYDLTTNKIYIDRSKSGVQINNKFSELNEQPVTRNADGSISLHLYVDRASVEAFTKGDTVLGANQIFPAPQSLGLQVVSEGGDSKADITLYPIKSVWTDKQKVNKPLEIVQVSPKEVRLNVGDSTTLTAYVMPGNVSQALDWSINDESLASITKDPESNSLKIVAKKAGTLTVTVKSHEDPSLSKTYKITILKNNFKTNIKDLKPLSGNWYVDDQDLHDENVSSNDYIMSPTKVSSSEYDMNLDVKYQKGLVNIFFASANEDPNGAYSLQLGGDKTLRLFRFYGDTITTTDLPAALNDGKLHHVAIHKTQNAVKVTIDGKEAMDYTFDKVDPGFNSAYVGLGLWDGAADFQNLYVKAATENDDNSSSSIDFNDQEIPNVSTDDNNSIIEKPSETVKTVVFTAKS

SEQ ID NO: 8 - protein, 859 aa, synthetic construct
DTQSPVNIEQKNKSAELIKQNSDISTSAQQHNKNANGKTEDTSTQSTSTDLQNTNGKTEDTSTQSTSTDLQNTNTQKSFKNQSQEPESSTKAGEVKTLKDFTFSQNGKWSEQKDGIHSDARGQGDSFAYTKVKGDNFMYSADVVFQTNQGAAAITFRDNNDPDNKDGYAVNVDASSHKAKFWRWHDNKDYQLIDERDVKQTADNTYNLKVVANGHWLEYFVNDVLVASNGDYTLQKGDKGQPSVTNNGYFGLLNWNSNVIFKNVKYTKLDQSFTPLVSDITVTSDKGKVEEKGQFSPEQPIYIQYVDNDASTVNLKVKTDSPKAKVVAYDLNNNAYTDLKNIPVQVGANYLTVVSEVTASDGTKVESVYRINVHRLHPNENYYNELYRDQYHFSVKEGWSNDPNGLVYFNGKYHMFYQFYDDTIWGPMHWAHATSKDLIHWKNEPIALYPDANGAMFSGSIVVDKGNTSGLFDNDKGGLVALVTTDGNGQRIELAYSRDEGKTWDKLPNLVADWQKDPLQVQDFRDPKVFRWNDKWFMVLAGGPLRIYSSTNLQNWQVESEYSNINTECPDLYPIRANDGQLKWVLSRGGRFYKIGDFKEVNGKWSFIPDEAYKDQDGIMNFGKDSYAAMTYYQHSFGTEKDPTLPDIIEENWMNNWDYCNLVGNTVGQSFNGAYNLNLKVGLVKDGDKYLLTQTPIKAYEALRDNAHKVEYKDVTVTPNNDLFKNFKGDSYEIVSTFRPSKSTTKVGFNVRVGKGQATKVIYDLTTNKIYIDRSKSGVQINNKFSELNEQPVTRNADGSISLHLYVDRASVEAFTKGDTVLGANQIFPAPQSLGLQVVSEGGDSKADITLYPIKSVWT

SEQ ID NO: 9 - protein, 1259 aa, Lactobacillus amylovorus
DTQSPVNIEQKNKSAELIKQNSDISASAQQHNKNANGKTEDTSTQSTSTDLQNTNTQKSFKNQSQEPESSTKAGEVKTLKDFTFSQNGKWSEQKDGIHSDARGQGDSFAYTKVKGDNFMYSADVVFQTNQGAAAITFRGNNDPNNKDGYAVNVDASSHKAKFWRWHDNKDYQLIDERDVKQTADNTYNLKVVANGHWLEYFVNDVLVASNGDYTLQKGDKGQPSVTNNGYFGLLNWNSNVIFKNVKYTKLDQSFTPLVSDITVTSDKGKVEEKGQFSPEQPIYIQYVDNDASTVNLKVKTDSPKAKVVAYDLNNNAYTDLKNIPVQVGANYLTVVSEVTASDGTKVESVYRINVHRLHPNENYYNELYRDQYHFSVKEGWSNDPNGLVYFNGKYHMFYQFYDDTIWGPMHWAHATSKDLIHWKNEPIALYPDANGAMFSGSIVVDKGNTSGLFDNDKGGLVALVTTDGNGQRIELAYSRDEGKTWNKLPNLVADWQKDPLQVQDFRDPKVFRWNDKWFMVLAGGPLRIYSSTNLQNWQVESEYSNINTECPDLYPIRANDGQLKWVLSRGGRFYKIGDFKEINGKWIFIPDEAYKDQDGIMNFGKDSYAAMTYYQHSFGTEKDPTLPDIIEENWMNNWDYCNLVGNTVGQSFNGTYNLNLKVGLVKDGDKYLLTQTPIKAYEALRDNAHKVEYKDVTVTPNNDLFKNFKGDSYEIVSTFRPSKSTTKVGFNVRVGKGQATKVIYDLTTNKIYIDRSKSGVQINNKFSELNEQPVTRNADGSISLHLYVDRASVEAFTKGDTVLGANQIFPAPQSLGLQVVSEGGDSKADITLYPMKSVWTDKQKVNKPLEIVQVSPKEVRLNVGDSTTLTAYVMPGNVSQALDWSVNDESLASITKDPESNSLKIVAKKTGTLTVTVKSHEDPSLSKTYKITILKNNFKTNIKNLKPLSGDWYINDKDLHDENVSSNDYIMSPTKIPSSEYDINLDVKYQKGLVNIFFASANEDPNGAYSLQLGGDKTLRLFRFYGDTITTTDLPAALNDGKLHHVAIHKTQKTVKVTVDGKTVMDYTFNKVDPGFNDAYIGLGLWDGTVDFQNLYVKTPTKNSDNSSSIDINDQGIPSISTDDNSSIIKKASENIQPIVFKTKILMHNAFVYNDTGKHIVKIILKAGSVLKVGKIKFINNKRYYQLDNDKYIKAANIDAFVRRLRRNAFVYNHIGKHIKNSLIRKGKKVKTYGSPVVIKGIKYYIVGNNRYIKAVNFM

SEQ ID NO: 10 - protein, 1145 aa, synthetic construct
DTQSPVNIEQKNKSAELIKQNSDISASAQQHNKNANGKTEDTSTQSTSTDLQNTNTQKSFKNQSQEPESSTKAGEVKTLKDFTFSQNGKWSEQKDGIHSDARGQGDSFAYTKVKGDNFMYSADVVFQTNQGAAAITFRGNNDPNNKDGYAVNVDASSHKAKFWRWHDNKDYQLIDERDVKQTADNTYNLKVVANGHWLEYFVNDVLVASNGDYTLQKGDKGQPSVTNNGYFGLLNWNSNVIFKNVKYTKLDQSFTPLVSDITVTSDKGKVEEKGQFSPEQPIYIQYVDNDASTVNLKVKTDSPKAKVVAYDLNNNAYTDLKNIPVQVGANYLTVVSEVTASDGTKVESVYRINVHRLHPNENYYNELYRDQYHFSVKEGWSNDPNGLVYFNGKYHMFYQFYDDTIWGPMHWAHATSKDLIHWKNEPIALYPDANGAMFSGSIVVDKGNTSGLFDNDKGGLVALVTTDGNGQRIELAYSRDEGKTWNKLPNLVADWQKDPLQVQDFRDPKVFRWNDKWFMVLAGGPLRIYSSTNLQNWQVESEYSNINTECPDLYPIRANDGQLKWVLSRGGRFYKIGDFKEINGKWIFIPDEAYKDQDGIMNFGKDSYAAMTYYQHSFGTEKDPTLPDIIEENWMNNWDYCNLVGNTVGQSFNGTYNLNLKVGLVKDGDKYLLTQTPIKAYEALRDNAHKVEYKDVTVTPNNDLFKNFKGDSYEIVSTFRPSKSTTKVGFNVRVGKGQATKVIYDLTTNKIYIDRSKSGVQINNKFSELNEQPVTRNADGSISLHLYVDRASVEAFTKGDTVLGANQIFPAPQSLGLQVVSEGGDSKADITLYPMKSVWTDKQKVNKPLEIVQVSPKEVRLNVGDSTTLTAYVMPGNVSQALDWSVNDESLASITKDPESNSLKIVAKKTGTLTVTVKSHEDPSLSKTYKITILKNNFKTNIKNLKPLSGDWYINDKDLHDENVSSNDYIMSPTKIPSSEYDINLDVKYQKGLVNIFFASANEDPNGAYSLQLGGDKTLRLFRFYGDTITTTDLPAALNDGKLHHVAIHKTQKTVKVTVDGKTVMDYTFNKVDPGFNDAYIGLGLWDGTVDFQNLYVKTPTKNSDNSSSIDINDQGIPSISTDDNSSIIKKASENIQPIVFKTKI

SEQ ID NO: 11 - protein, 1145 aa, synthetic construct
DTQSPVNIEQKNKSAELIKQNSDISASAQQHNKNANGKTEDTSTQSTSTDLQNTNTQKSFKNQSQEPESSTKAGEVKTLKDFTFSQNGKWSEQKDGIHSDARGQGDSFAYTKVKGDNFMYSADVVFQTNQGAAAITFRGNNDPNNKDGYAVNVDASSHKAKFWRWHDNKDYQLIDERDVKQTADNTYNLKVVANGHWLEYFVNDVLVASNGDYTLQKGDKGQPSVTNNGYFGLLNWNSNVIFKNVKYTKLDQSFTPLVSDITVTSDKGKVEEKGQFSPEQPIYIQYVDNDASTVNLKVKTDSPKAKVVAYDLNNNAYTDLKNIPVQVGANYLTVVSEVTASDGTKVESVYRINVHRLHPNENYYNELYRDQYHFSVKEGWSNDPNGLVYFNGKYHMFYQFYDDTIWGPMHWAHATSKDLIHWKNEPIALYPDANGAMFSGSIVVDKGNTSGLFDNDKGGLVALVTTDGNGQRIELAYSRDEGKTWNKLPNLVADWQKDPLQVQDFRDPKVFRWNDKWFMVLAGGPLRIYSSTNLQNWQVESEYSNINTECPDLYPIRANDGQLKWVLSRGGRFYKIGDFKEINGKWIFIPDEAYKDQDGIMNFGKDSYAAMTYYQHSFGTEKDPTLPDIIEENWMNNWDYCNLVGNTVGQSFNGAYNLNLKVGLVKDGDKYLLTQTPIKAYEALRDNAHKVEYKDVTVTPNNDLFKNFKGDSYEIVSTFRPSKSTTKVGFNVRVGKGQATKVIYDLTTNKIYIDRSKSGVQINNKFSELNEQPVTRNADGSISLHLYVDRASVEAFTKGDTVLGANQIFPAPQSLGLQVVSEGGDSKADITLYPMKSVWTDKQKVNKPLEIVQVSPKEVRLNVGDSTTLTAYVMPGNVSQALDWSVNDESLASITKDPESNSLKIVAKKTGTLTVTVKSHEDPSLSKTYKITILKNNFKTNIKNLKPLSGDWYINDKDLHDENVSSNDYIMSPTKIPSSEYDINLDVKYQKGLVNIFFASANEDPNGAYSLQLGGDKTLRLFRFYGDTITTTDLPAALNDGKLHHVAIHKTQKTVKVTVDGKTVMDYTFNKVDPGFNDAYIGLGLWDGTVDFQNLYVKTPTKNSDNSSSIDINDQGIPSISTDDNSSIIKKASENIQPIVFKTKI

SEQ ID NO: 12 - protein, 1279 aa, Lactobacillus crispatus
DTQSPVNIEQKNKSAELIKQNSDISTSAQQHNKNANGKTEDTSTQSTSTDLQNTNGKTEDTSTQSTSTDLQNTNTQKSFKNQSQEPESSTKAGEVKTLKDFTFSQNGKWSEQKDGIHSDARGQGDSFAYTKVKGDNFMYSADVVFQTNQGAAAITFRDNNDPDNKDGYAVNVDASSHKAKFWRWHDNKDYQLIDERDVKQTADNTYNLKVVANGHWLEYFVNDVLVASNGDYTLQKGDKGQPSVTNNGYFGLLNWNSNVIFKNVKYTKLDQSFTPLVSDITVTSDKGKVEEKGQFSPEQPIYIQYVDNDASTVNLKVKTDSPKAKVVAYDLNNNAYTDLKNIPVQVGANYLTVVSEVTASDGTKVESVYRINVHRLHPNENYYNELYRDQYHFSVKEGWSNDPNGLVYFNGKYHMFYQFYDDTIWGPMHWAHATSKDLIHWKNEPIALYPDANGAMFSGSIVVDKGNTSGLFDNDKGGLVALVTTDGNGQRIELAYSRDEGKTWNKLPNLVADWQKDPLQVQDFRDPKVFRWNDKWFMVLAGGPLRIYSSTNLQNWQVESEYSNINTECPDLYPIRANDGQLKWVLSRSGRFYKIGDFKEVNGKWSFIPDEAYKDQDGIMNFGKDSYAAMTYYQHSFGTEKDPTLPDIIEENWMNNWDYCNLVGNTVGQSFNGTYNLNLKVGLVKDGDKYLLTQTPIKAYETLRDNAHKVEYKDVTVTPNNDLFKNFKGDSYEIVSTFRPSKSTTKVGFNVRVGKGQATKVIYDLTTNKIYIDRSKSGVQINNKFSELNEQPVTRNADGSISLHLYVDRASVEAFTKGDTVLGANQIFPAPQSLGLQVVSEGGDSKADITLYPIKSVWTDKQKVNKPLEIVQVSPKEVRLNVGDSTTLTAYVMPGNVSQALDWSVNDESLASIAKDPESNSLKIVAKKAGTLTVTVKSHEDPSLSKTYKITILKNNFKTNIKDLKPLSGNWYVDDQDLHDENVSSNDYIMSPTKVSSSEYDMNLDVKYQKGLVNIFFASANEDPNGAYSLQLGGDKTLRLFRFYGDTITTTDLPAALNDGKLHHVAIHKTQNAVKVTIDGKEAMDYTFDKVDPGFNSAYVGLGLWDGAADFQNLYVKAATENDDNSSSSIDFNDQEIPNVSTDDNNSIIEKPSETVKTVVFTAKSLMHNAFVYDNQGKRIEKIVLKAGSVLKVGHIKLINHKRYYQLDNGKYIKAGNIDAYVRKLRRNAFVYNRAGKHIKKSLIRKGKKVKTYGSPVVIKGKKYYVVGKNRYIKAVNFM

SEQ ID NO: 13 - protein, 1165 aa, synthetic construct
DTQSPVNIEQKNKSAELIKQNSDISTSAQQHNKNANGKTEDTSTQSTSTDLQNTNGKTEDTSTQSTSTDLQNTNTQKSFKNQSQEPESSTKAGEVKTLKDFTFSQNGKWSEQKDGIHSDARGQGDSFAYTKVKGDNFMYSADVVFQTNQGAAAITFRDNNDPDNKDGYAVNVDASSHKAKFWRWHDNKDYQLIDERDVKQTADNTYNLKVVANGHWLEYFVNDVLVASNGDYTLQKGDKGQPSVTNNGYFGLLNWNSNVIFKNVKYTKLDQSFTPLVSDITVTSDKGKVEEKGQFSPEQPIYIQYVDNDASTVNLKVKTDSPKAKVVAYDLNNNAYTDLKNIPVQVGANYLTVVSEVTASDGTKVESVYRINVHRLHPNENYYNELYRDQYHFSVKEGWSNDPNGLVYFNGKYHMFYQFYDDTIWGPMHWAHATSKDLIHWKNEPIALYPDANGAMFSGSIVVDKGNTSGLFDNDKGGLVALVTTDGNGQRIELAYSRDEGKTWNKLPNLVADWQKDPLQVQDFRDPKVFRWNDKWFMVLAGGPLRIYSSTNLQNWQVESEYSNINTECPDLYPIRANDGQLKWVLSRSGRFYKIGDFKEVNGKWSFIPDEAYKDQDGIMNFGKDSYAAMTYYQHSFGTEKDPTLPDIIEENWMNNWDYCNLVGNTVGQSFNGAYNLNLKVGLVKDGDKYLLTQTPIKAYETLRDNAHKVEYKDVTVTPNNDLFKNFKGDSYEIVSTFRPSKSTTKVGFNVRVGKGQATKVIYDLTTNKIYIDRSKSGVQINNKFSELNEQPVTRNADGSISLHLYVDRASVEAFTKGDTVLGANQIFPAPQSLGLQVVSEGGDSKADITLYPIKSVWTDKQKVNKPLEIVQVSPKEVRLNVGDSTTLTAYVMPGNVSQALDWSVNDESLASIAKDPESNSLKIVAKKAGTLTVTVKSHEDPSLSKTYKITILKNNFKTNIKDLKPLSGNWYVDDQDLHDENVSSNDYIMSPTKVSSSEYDMNLDVKYQKGLVNIFFASANEDPNGAYSLQLGGDKTLRLFRFYGDTITTTDLPAALNDGKLHHVAIHKTQNAVKVTIDGKEAMDYTFDKVDPGFNSAYVGLGLWDGAADFQNLYVKAATENDDNSSSSIDFNDQEIPNVSTDDNNSIIEKPSETVKTVVFTAKS